European Patent Specification EP 3 419 989 B1, published March 19, 2025. Title: REDOX LABELED OLIGONUCLEOTIDE PROBES AND THEIR USE. Applicant: Alere San Diego Inc. The sequence listing filed with the application follows.

SEQUENCE LISTING (17 sequences)

SEQ ID NO: 1 - DNA, 41 bp, Artificial Sequence
  artificial oligos
  misc_feature (27)..(27): N = deoxyribonucleotide conjugated to a redox moiety
aagcaattgaggagtgcctgattaatnatccctgggttttg

SEQ ID NO: 2 - DNA, 36 bp, Artificial Sequence
  artificial oligos
  misc_feature (21)..(21): N = deoxyribonucleotide conjugated to a redox moiety
gtctggctgtcagtaagtatnctagagtcccgtttt

SEQ ID NO: 3 - DNA, 41 bp, Artificial Sequence
  artificial oligos
  misc_feature (28)..(28): N = deoxyribonucleotide conjugated to a redox moiety
tcagctacaatcaagactactcgttaantaatgaatcctca

SEQ ID NO: 4 - DNA, 42 bp, Artificial Sequence
  artificial oligos
  misc_feature (28)..(28): N = deoxyribonucleotide conjugated to a redox moiety
gcacacttgtcacctacatttctgattngtggactctaacat

SEQ ID NO: 5 - DNA, 45 bp, Artificial Sequence
  artificial oligos
  misc_feature (28)..(28): N = T conjugated to a redox moiety
  misc_feature (30)..(30): N = modified naturally occurring amino acid
catcagcttttggagcttgagagtcatnangtttttgagcttcac

SEQ ID NO: 6 - DNA, 48 bp, Artificial Sequence
  artificial oligos
  misc_feature (32)..(32): N = T conjugated to a redox moiety
  misc_feature (33)..(33): N = modified naturally occurring amino acid
gaaccaagaagcattragcaaaacccagggannattaatcaggcactc

SEQ ID NO: 7 - DNA, 45 bp, Artificial Sequence
  artificial oligos
  misc_feature (17)..(17): N = T conjugated to a redox moiety
  misc_feature (22)..(22): N = T conjugated to a redox moiety
  misc_feature (29)..(29): N = T conjugated to a redox moiety
  misc_feature (30)..(30): N = modified naturally occurring amino acid
actgatgatattcagcnacaancaagacnntcgttaagtaatgaa

SEQ ID NO: 8 - DNA, 38 bp, Artificial Sequence
  artificial oligos
  misc_feature (6)..(6): N = deoxyribonucleotide conjugated to a redox moiety
  misc_feature (38)..(38): N = 2',3'dideoxycytidine residue
acccanggatcattaatcaggcactcctcaattgcttn

SEQ ID NO: 9 - DNA, 41 bp, Artificial Sequence
  artificial oligos
  misc_feature (15)..(15): N = deoxyribonucleotide conjugated to a redox moiety
  misc_feature (27)..(27): N = deoxyribonucleotide conjugated to a redox moiety
aataccgcgaggtgnagcaaatctatnaaatatgtcccagt

SEQ ID NO: 10 - DNA, 50 bp, Artificial Sequence
  artificial oligos
  misc_feature (15)..(15): N = deoxyribonucleotide conjugated to a redox moiety
  misc_feature (36)..(36): N = deoxyribonucleotide conjugated to a redox moiety
attttctctggatgntatgcccggtaaacagatgantattgatgccgatt

SEQ ID NO: 11 - DNA, 48 bp, Artificial Sequence
  artificial oligos
  misc_feature (15)..(15): N = deoxyribonucleotide conjugated to a redox moiety
  misc_feature (34)..(34): N = deoxyribonucleotide conjugated to a redox moiety
tcgaaaagaaacacncggatgaaatcgataagtntatacaaggattgg

SEQ ID NO: 12 - DNA, 35 bp, Artificial Sequence
  artificial oligos
cgtgctacaatggcatatacaatgagacgcaatac

SEQ ID NO: 13 - DNA, 32 bp, Artificial Sequence
  artificial oligos
ccggcttcatgctctcgagttgcagagaacaa

SEQ ID NO: 14 - DNA, 34 bp, Artificial Sequence
  artificial oligos
gtggtccagtttatcgttattaccaaaggttcag

SEQ ID NO: 15 - DNA, 32 bp, Artificial Sequence
  artificial oligos
ccgttcgcgcgcrgcatccgcatcaataatac

SEQ ID NO: 16 - DNA, 36 bp, Artificial Sequence
  artificial oligos
cgcctgcaagtcctaagacgccaatcgaaaagaaac

SEQ ID NO: 17 - DNA, 35 bp, Artificial Sequence
  artificial oligos
ctgcatctccgtggtatactaatacattgttttta